European Patent Specification EP 3 412 770 B1, published September 10, 2025. Title: Genetically-engineered cultured cell in which norovirus can be grown, and use thereof. Applicant: JAPAN AS REPRESENTED BY DIRECTOR-GENERAL OF NATIONAL INSTITUTE OF INFECTIOUS DISEASES DENKA COMPANY LIMITED. The sequence listing filed with the application follows.

SEQUENCE LISTING (16 sequences)

SEQ ID NO: 1 - DNA, 1014 bp, mouse
  CDS (1)..(1011)
atgcatttgtcactgctggtcccctttctcttctggatcacaggctgctgcacggctcaggatccagtcacaggtccagaggaggtgagcggtcaggagcagggctccttgacagtgcagtgccgatatacctcaggctggaaggattacaagaagtactggtgccgaggagcttattggaaatcatgtgagattcttgttgaaaccgataaatcagagcagctggtgaagaagaaccgtgtgtccatcagggacaaccagagagacttcatcttcacagtgaccatggaagacctgaggatgagcgatgctggcatttactggtgtggaattacaaaagctggacctgatcccatgtttaaagttgctgtgaacattggcccagcaatccaagtacccattacagtgccaaccatgccccccatcacctccaccaccaccatcttcacagtgacaaccacggtaaaagagaccagcatgtttccaacgctgaccggctactactctgataatgggcatggcggtggtgacagtggcggtggtgaagatggcgtcggtgatgggtttctggatctcagtgtgctcctcccagtcatctctgcagtcctgttgcttctcctgttggtggcctcgctctttgcttggaggatggtgaggagacagaagaaagctgctgggccaccatcagagcaggcacagtctctggagggtgatctctgttatgcagacctgtccctgaagcagcccagaacctcccctggctcctcttggaaaaagggctcctccatgtcctcctctggcaaggaccaccaagaggaagtggaatatgtcaccatggctccctttcccagggaggaggtttcatatgccgctctgactttggctggcttgggtcaggagcctacttatggcaatactggctgccccatcacccatgttcccaggacaggccttgaagaggagaccacagagtacagcagcatcaggaggcccttgcctgcagccatgcattaa

SEQ ID NO: 2 - protein, 337 aa, mouse
MHLSLLVPFLFWITGCCTAQDPVTGPEEVSGQEQGSLTVQCRYTSGWKDYKKYWCRGAYWKSCEILVETDKSEQLVKKNRVSIRDNQRDFIFTVTMEDLRMSDAGIYWCGITKAGPDPMFKVAVNIGPAIQVPITVPTMPPITSTTTIFTVTTTVKETSMFPTLTGYYSDNGHGGGDSGGGEDGVGDGFLDLSVLLPVISAVLLLLLLVASLFAWRMVRRQKKAAGPPSEQAQSLEGDLCYADLSLKQPRTSPGSSWKKGSSMSSSGKDHQEEVEYVTMAPFPREEVSYAALTLAGLGQEPTYGNTGCPITHVPRTGLEEETTEYSSIRRPLPAAMH

SEQ ID NO: 3 - DNA, 1014 bp, mouse
  CDS (1)..(1011)
atgcatttgtcattgctggtcccctttctcttctggatcacaggctgctgcacggctgaggatccagtcacaggtccagaggaggtgagcggtcaggagcagggctccttgacagtgcagtgccgatatacctcaggctggaaggattacaagaagtactggtgccaaggagttcctcagagatcatgtaagactcttgttgaaaccgatgcatcagagcagctggtgaagaagaaccgtgtgtccatcagggacaaccagagagacttcatcttcacagtgaccatggaggatctgaggatgagcgatgctggcatttactggtgtggaattacgaaaggtggacttgatcccatgtttaaagttactgtgaacattggcccagcaatccaagtacccattacagtgccaaccatgccccccatcacctccaccaccaccatcttcacagtgacaaccacagtaaaagagaccagcatgtttccaacgctgactagctactactctgataacgggcatggcggtggtgacagtggcggtggtgaagatggcgtcggtgatgggtttctggatctcagtgtgctcctcccagtcatctctgcagtcctgttgcttctcctgttggtggcctcgctctttgcttggaggatggtgaggagacagaagaaagctgctgggccaccatcagagcaggcacagtctctggagggtgatctctgttatgcagacctgtccctgaagcagcccagaacctcccctggctcctcttggaaaaagggctcctccatgtcctcctctggcaaggaccaccaagaggaagtggaatatgtcaccatggctccctttcccagggaggaggtttcatatgccgctctgactttggccggcttgggtcaggagcctacttatggcaatactggctgccccatcacccacgttcccaggacaggccttgaagaggagaccacagagtacagcagcatcaggaggcccttgcctgcagccatgccttaa

SEQ ID NO: 4 - protein, 337 aa, mouse
MHLSLLVPFLFWITGCCTAEDPVTGPEEVSGQEQGSLTVQCRYTSGWKDYKKYWCQGVPQRSCKTLVETDASEQLVKKNRVSIRDNQRDFIFTVTMEDLRMSDAGIYWCGITKGGLDPMFKVTVNIGPAIQVPITVPTMPPITSTTTIFTVTTTVKETSMFPTLTSYYSDNGHGGGDSGGGEDGVGDGFLDLSVLLPVISAVLLLLLLVASLFAWRMVRRQKKAAGPPSEQAQSLEGDLCYADLSLKQPRTSPGSSWKKGSSMSSSGKDHQEEVEYVTMAPFPREEVSYAALTLAGLGQEPTYGNTGCPITHVPRTGLEEETTEYSSIRRPLPAAMP

SEQ ID NO: 5 - DNA, 666 bp, mouse
  CDS (1)..(663)
atgtggcagttctctgctctactcctattcttcctcccaggctgctgcactgctcagaatccagtcacaggtccagaggaggtgagcggtcaggagcagggctccttgacagtgcagtgccaatatacctcagactggaaggattacaagaagtactggtgccaaggagttcctcagaaatcatgtgtttttcttattgaaactgataaatcagagcagttggtgaagaagaaccgtgtgtccatcagggacaaccaaagagagttcatcttcacagtgatcatggaggatctgaggatgagcgatgctggcatttactggtgtggaattacgaaagctggatatgatcccgtctttaaagttaatgtgagcattaacccagccccaaaaagttcaatgatgaccaccacagccacagttctgaaatccatacaaccaagcgctgagaacactggcaaggaacaagtgactcagagcaaagaagtgactcagagcaggccccacaccaggtccctgctgagcagcatctacttcctgctgatggtctttgtggagttacccctgctcctgagcatgctcagtgctgtcctctgggtgaccaggcctcagagatgctttgggagaggtgaaaatgacctggtgaagacccatagtcctgttgcctag

SEQ ID NO: 6 - protein, 221 aa, mouse
MWQFSALLLFFLPGCCTAQNPVTGPEEVSGQEQGSLTVQCQYTSDWKDYKKYWCQGVPQKSCVFLIETDKSEQLVKKNRVSIRDNQREFIFTVIMEDLRMSDAGIYWCGITKAGYDPVFKVNVSINPAPKSSMMTTTATVLKSIQPSAENTGKEQVTQSKEVTQSRPHTRSLLSSIYFLLMVFVELPLLLSMLSAVLWVTRPQRCFGRGENDLVKTHSPVA

SEQ ID NO: 7 - DNA, 912 bp, Artificial Sequence
  MuRaw_d102
  CDS (1)..(909)
atgcatttgtcattgctggtcccctttctcttctggatcacaggctgctgcaagtactggtgccaaggagttcctcagagatcatgtaagactcttgttgaaaccgatgcatcagagcagctggtgaagaagaaccgtgtgtccatcagggacaaccagagagacttcatcttcacagtgaccatggaggatctgaggatgagcgatgctggcatttactggtgtggaattacgaaaggtggacttgatcccatgtttaaagttactgtgaacattggcccagcaatccaagtacccattacagtgccaaccatgccccccatcacctccaccaccaccatcttcacagtgacaaccacagtaaaagagaccagcatgtttccaacgctgactagctactactctgataacgggcatggcggtggtgacagtggcggtggtgaagatggcgtcggtgatgggtttctggatctcagtgtgctcctcccagtcatctctgcagtcctgttgcttctcctgttggtggcctcgctctttgcttggaggatggtgaggagacagaagaaagctgctgggccaccatcagagcaggcacagtctctggagggtgatctctgttatgcagacctgtccctgaagcagcccagaacctcccctggctcctcttggaaaaagggctcctccatgtcctcctctggcaaggaccaccaagaggaagtggaatatgtcaccatggctccctttcccagggaggaggtttcatatgccgctctgactttggccggcttgggtcaggagcctacttatggcaatactggctgccccatcacccacgttcccaggacaggccttgaagaggagaccacagagtacagcagcatcaggaggcccttgcctgcagccatgccttaa

SEQ ID NO: 8 - protein, 303 aa, Artificial Sequence
  Synthetic Construct
MHLSLLVPFLFWITGCCKYWCQGVPQRSCKTLVETDASEQLVKKNRVSIRDNQRDFIFTVTMEDLRMSDAGIYWCGITKGGLDPMFKVTVNIGPAIQVPITVPTMPPITSTTTIFTVTTTVKETSMFPTLTSYYSDNGHGGGDSGGGEDGVGDGFLDLSVLLPVISAVLLLLLLVASLFAWRMVRRQKKAAGPPSEQAQSLEGDLCYADLSLKQPRTSPGSSWKKGSSMSSSGKDHQEEVEYVTMAPFPREEVSYAALTLAGLGQEPTYGNTGCPITHVPRTGLEEETTEYSSIRRPLPAAMP

SEQ ID NO: 9 - DNA, 810 bp, Artificial Sequence
  MuRaw_d204
  CDS (1)..(807)
atgcatttgtcattgctggtcccctttctcttctggatcacaggctgctgcaaccagagagacttcatcttcacagtgaccatggaggatctgaggatgagcgatgctggcatttactggtgtggaattacgaaaggtggacttgatcccatgtttaaagttactgtgaacattggcccagcaatccaagtacccattacagtgccaaccatgccccccatcacctccaccaccaccatcttcacagtgacaaccacagtaaaagagaccagcatgtttccaacgctgactagctactactctgataacgggcatggcggtggtgacagtggcggtggtgaagatggcgtcggtgatgggtttctggatctcagtgtgctcctcccagtcatctctgcagtcctgttgcttctcctgttggtggcctcgctctttgcttggaggatggtgaggagacagaagaaagctgctgggccaccatcagagcaggcacagtctctggagggtgatctctgttatgcagacctgtccctgaagcagcccagaacctcccctggctcctcttggaaaaagggctcctccatgtcctcctctggcaaggaccaccaagaggaagtggaatatgtcaccatggctccctttcccagggaggaggtttcatatgccgctctgactttggccggcttgggtcaggagcctacttatggcaatactggctgccccatcacccacgttcccaggacaggccttgaagaggagaccacagagtacagcagcatcaggaggcccttgcctgcagccatgccttaa

SEQ ID NO: 10 - protein, 269 aa, Artificial Sequence
  Synthetic Construct
MHLSLLVPFLFWITGCCNQRDFIFTVTMEDLRMSDAGIYWCGITKGGLDPMFKVTVNIGPAIQVPITVPTMPPITSTTTIFTVTTTVKETSMFPTLTSYYSDNGHGGGDSGGGEDGVGDGFLDLSVLLPVISAVLLLLLLVASLFAWRMVRRQKKAAGPPSEQAQSLEGDLCYADLSLKQPRTSPGSSWKKGSSMSSSGKDHQEEVEYVTMAPFPREEVSYAALTLAGLGQEPTYGNTGCPITHVPRTGLEEETTEYSSIRRPLPAAMP

SEQ ID NO: 11 - DNA, 912 bp, Artificial Sequence; identical to SEQ ID NO: 7
  MuRAW_d120v
  CDS (1)..(909)

SEQ ID NO: 12 - protein, 303 aa, Artificial Sequence; identical to SEQ ID NO: 8
  Synthetic Construct

SEQ ID NO: 13 - DNA, 1014 bp, Artificial Sequence
  MuRAW_dcpd
  CDS (1)..(684)
atgcatttgtcattgctggtcccctttctcttctggatcacaggctgctgcacggctgaggatccagtcacaggtccagaggaggtgagcggtcaggagcagggctccttgacagtgcagtgccgatatacctcaggctggaaggattacaagaagtactggtgccaaggagttcctcagagatcatgtaagactcttgttgaaaccgatgcatcagagcagctggtgaagaagaaccgtgtgtccatcagggacaaccagagagacttcatcttcacagtgaccatggaggatctgaggatgagcgatgctggcatttactggtgtggaattacgaaaggtggacttgatcccatgtttaaagttactgtgaacattggcccagcaatccaagtacccattacagtgccaaccatgccccccatcacctccaccaccaccatcttcacagtgacaaccacagtaaaagagaccagcatgtttccaacgctgactagctactactctgataacgggcatggcggtggtgacagtggcggtggtgaagatggcgtcggtgatgggtttctggatctcagtgtgctcctcccagtcatctctgcagtcctgttgcttctcctgttggtggcctcgctctttgcttggaggatggtgaggagacagaagaaagctgctgggccaccataagagcaggcacagtctctggagggtgatctctgttatgcagacctgtccctgaagcagcccagaacctcccctggctcctcttggaaaaagggctcctccatgtcctcctctggcaaggaccaccaagaggaagtggaatatgtcaccatggctccctttcccagggaggaggtttcatatgccgctctgactttggccggcttgggtcaggagcctacttatggcaatactggctgccccatcacccacgttcccaggacaggccttgaagaggagaccacagagtacagcagcatcaggaggcccttgcctgcagccatgccttaa

SEQ ID NO: 14 - protein, 228 aa, Artificial Sequence
  Synthetic Construct
MHLSLLVPFLFWITGCCTAEDPVTGPEEVSGQEQGSLTVQCRYTSGWKDYKKYWCQGVPQRSCKTLVETDASEQLVKKNRVSIRDNQRDFIFTVTMEDLRMSDAGIYWCGITKGGLDPMFKVTVNIGPAIQVPITVPTMPPITSTTTIFTVTTTVKETSMFPTLTSYYSDNGHGGGDSGGGEDGVGDGFLDLSVLLPVISAVLLLLLLVASLFAWRMVRRQKKAAGPP

SEQ ID NO: 15 - DNA, 386 bp, Artificial Sequence
  RuRaw_d120vC term
  CDS (1)..(384)
atgcatttgtcattgctggtcccctttctcttctggatcacaggctgctgcacggctgaggatccagtcacaggtccagaggaggtgagcggtcaggagcagggctccttgacagtgcagtgccgatatacctcaggctggaaggattacaagaagtactggtgccaaggagttcctcagagatcatgtaagactcttgttgaaaccgatgcatcagagcagctggtgaagaagaaccgtgtgtccatcagggacaaccagagagacttcatcttcacagtgaccatggaggatctgaggatgagcgatgctggcatttactggtgtggaattacgaaaggtggacttgatcccatgtttaaagttactgtgaacattggcccagg

SEQ ID NO: 16 - protein, 128 aa, Artificial Sequence
  Synthetic Construct
MHLSLLVPFLFWITGCCTAEDPVTGPEEVSGQEQGSLTVQCRYTSGWKDYKKYWCQGVPQRSCKTLVETDASEQLVKKNRVSIRDNQRDFIFTVTMEDLRMSDAGIYWCGITKGGLDPMFKVTVNIGP